European Patent Specification EP 3 748 005 B1, published May 6, 2026. Title: 催化谷氨酰胺合成靛蓝获得蓝色花卉的转基因方法. Applicant: 天津大学；中国科学院微生物研究所. The sequence listing filed with the application follows.

SEQUENCE LISTING (11 sequences)

SEQ ID NO: 1 - DNA, 675 bp, 人工序列(Artificial Sequence)
atgaagatttacagaatttatatggaccgcccgctttcacaggaagaaaatgaacggttcatgtctttcatatcacctgaaaaacgggagaaatgccggagattttatcataaagaagatgctcaccgcaccctgctgggagatgtgctcgttcgctcagtcataagcaggcagtatcagttggacaaatccgatatccgctttagcacgcaggaatacgggaagccgtgcatcactgatcttcccgacgctcatttcaacatttctcactccggccgctgggtcattggtgcgtttgattcacagccgatcggcatagatatcgaaaaaacgaaaccgatcagccttgagatcgccaagcgcttcttttcaaaaacagagtacagcgaccttttagcaaaagacaaggacgagcgaacagactatttttatcatctatggtcaatgaaagagagctttatcaaacaggaaggcaaaggcttatcgcttccgcttgattccttttcagtgcgcctgcatcaggacggacaagtatccattgagcttccggacagccattccccatgctatatcaaaacgtatgaggtcgatcccggctacaaaatggctgtatgcgccgcacaccctgatttccccgaggatatcacaatggtgtcgtacgaagagcttttatag

SEQ ID NO: 2 - protein, 224 aa, 枯草芽孢杆菌(Bacillus subtilis)
MKIYRIYMDRPLSQEENERFMSFISPEKREKCRRFYHKEDAHRTLLGDVLVRSVISRQYQLDKSDIRFSTQEYGKPCITDLPDAHFNISHSGRWVIGAFDSQPIGIDIEKTKPISLEIAKRFFSKTEYSDLLAKDKDERTDYFYHLWSMKESFIKQEGKGLSLPLDSFSVRLHQDGQVSIELPDSHSPCYIKTYEVDPGYKMAVCAAHPDFPEDITMVSYEELL

SEQ ID NO: 3 - DNA, 3852 bp, 人工序列(Artificial Sequence)
atgacccttcaagaaaccagcgttctggaaccgaccctgcgcggaacgaccaccctgccggatctgctggcaaaacgggttgcagaacatccggaagcaaccgcagttgcatatcgcgatgaaaaactgacctatcgtgaactggcaagccgtagcagcgcactggcagaatatctgcgtcatctgggtgttagcaccgatgattgtgttggtctgtttgttgaaccgagcattgatctgatggttggtgcatggggtattctgagcgcaggtgcagcatatctgccgctgagcccggaatatccggaagatcgcctgcgctatatgattgaaaatagccaggcaaaaattattctggcacagcagcgcctggttacccgcctgcgcgaactggcaccgcaggatgttcgtgttgttaccctgcgcgaaagcgaagcatttgttctgccggaaggtcaggttgcaccggcaattgaaggtgcacgtccggatagcctggcttatgttatctataccagcggtagcaccggtaaaccgaaaggtgttatgattgaacatcatagcattgttagccagctgggttggctgcgcgaaacctatggtattgatcgtagcaaaaccattttacagaaaaccccgatgagctttgatgcagcacagtgggaaattctgagcccggcaaatggtgcaaccgttgttatgggtgcaccgggtgtttatgcagatccggaaggtctgattgaaaccattgttaaatatggtgttaccaccctccagtgtgttccgaccctgctgcaaggtctgctggataccgaaaaatttccggaatgtaccagcttgcagcagatttttagcggtggtgaagcactgagccgcctgctggcaattcagaccacccaggaaatgccgggtcgcgcactgattaatgtttatggtccgaccgaatgtaccattaatagcagcagctatgcagttgatccggcagaactgggtgaagcaccgcagagcattagcattggtgcaccggttgcagataccgaatatcatattctgggtaaagaggacctgaaaccggttggtgttggtgaaattggtgaactgtatattggtggtggtcagctggcacgcggttatctgcatcgcccggatctgaccgcagaacgctttctggaaattgaagttaccgaaggtgcaggtccggttcgcctgtacaagaccggcgacctgggtcagtggaatccggatggaaccgttcagtttgcaggtcgcgcagataatcaggttaaactgcgcggttatcgtgttgaactggatgaaattagcctggcaattgaaaatcatgattgggttcgtaatgcagcagttattgttaaaaatgatggtcgtaccggttttcagaatctgattgcatgtgttgaactgagcgaaaaagaagcagcactgatggatcagggtaatcatggtagccatcatgcaagcaaaaaatccaaattgcaggttaaagcacagctgagcaatccgggtctgcgcgatgatgcggatctggcagccagagttgcttacgatctgccgggtgcagaaccgaccccggaacagcgtagccgtgtttttgcaaggaaaacctatcgcttttatgaaggtggtgcagttaccgaagccgacctgctggcactgctgggtggtcaggttccggcagcatatagccgtaaagcagctgacctggcaccggcagaactgggtcagattctgcgttggtttggtcagtatctgagcgaagaacgcctgctgccgaaatatggttatgcatcgccaggtgcactgtatgcaacccagctgtattttgaactggaaggtgttggtggtctgcaaccgggttattattattatcagccgcagcgccatcagctggttctgattagcgaaaaagcagcaaccggtcgtccgaccgcacatattcattttattggtaaacgcggtggtattgaaccggtttacaaaaacaatattcaggaagttctggaaattgaaaccggtcatattgttggtctgtttgaacaggttctgccggcctacggtctggatattcgtgatctggcctacgaaccggcagttcgcgatctgctggatgttccggaagaagatttttatctgggaacgtttgaactggttccgcataccggtcgtcgtgaagatcatgcagaagtttatgttcagactcacggtagcaaagttgcaaatctgccggaaggtcagtatcgctatgcagatggcacgctgacccgctttagcgatgatattgttctgaaaaaacaggttattgcaattaatcagagcgtttatcaggcagcctcctttggtattagcgttattagccgcgcaccggaagagtggatgcattatgttaccctgggcaagaaactccagcatctgatgatgaatggtctgggtctgggttttatgagcagcggttatagcagcaaaaccggtaatccgctgccggcaagccgtcgcattgatagcgttctacaagcaaatggtgttgaaagcggtccgagctatttctttgttggtggtcgtgttagcgatgaacagctgggtcatgaaggtatgcgtgaagatagcgttcacatgcgcggtccggcagaactgattcgcgatgatctggttagctttctgccggattatatgattccgaatcgtgttgttgtttttgaacgcctgccgctgagcgcaaatgggaagattgatgcaaaagcactggcagcaagcgatcaggttaatgcagaactggttgaacgcccgtttgttgcaccgcgtaccgaaaccgaaaaagaaattgcagaagtttgggcaaaaagcctgcgtcgcgaaagcgttagcgttcaggatgatttctttgaaagcggtggtaatagcctgattgcagttggtctgattcgcgaactgaatagccgcctgggtgttagcctgccgctacagagcgttctggaaagcccgaccgttgaaaaactgagccgtcgcctggaacgcgaagttgcacaggaaagcagccgcctggttcgccttcacgcagaaaccggtaaagatcgtccggttctgtgttggccgggtctgggtggttatccgatgaatctgcgtaccctggcaggtgaaattggtctgggtcgtagcttttatggtattcaggcacatggtattaacgaaggtgaagcaccgtatgcaaccattaccgaaatggcaaaagcagatattgaagcaattaaagaattgcaaccgaaaggtccgtataccctgtggggttatagctttggtgcgcgtgttgcatttgaaaccgcatatcagctggaacaggcaggtgaaaaagttgataatctgtttctgattgcaccgggtagcccgaccgttcgcgcagaaaatggtaaagtttatggtcgcgaagccagttttgcaaatcgcgcatataccaccattctgtttagcgtttttaccggaactattagcggtccggatctggaaaaatgtctggaaagcgcaaccgatgaagaaagttttgcaggttttattagcgaactgaaaggtattgatgttgatctggcaaaacgtattattagcgttgttggtcagacctatgaatttgaatatagctttcgcgaactggcagaacgtaccctggcagcaccggttaccatttttaaagcacgcggcgatgattatagctttattgaaaatagcaatggttatagcgcagaaccgccgaccgttattgatctggatgcagatcattatagcctgctgcgtaccccggatattggtgaactggttaaacatattcgctatctgctgggtgaataa

SEQ ID NO: 4 - protein, 1283 aa, 淡紫灰链霉菌(Streptomyces lavendulae)
MTLQETSVLEPTLRGTTTLPDLLAKRVAEHPEATAVAYRDEKLTYRELASRSSALAEYLRHLGVSTDDCVGLFVEPSIDLMVGAWGILSAGAAYLPLSPEYPEDRLRYMIENSQAKIILAQQRLVTRLRELAPQDVRVVTLRESEAFVLPEGQVAPAIEGARPDSLAYVIYTSGSTGKPKGVMIEHHSIVSQLGWLRETYGIDRSKTILQKTPMSFDAAQWEILSPANGATVVMGAPGVYADPEGLIETIVKYGVTTLQCVPTLLQGLLDTEKFPECTSLQQIFSGGEALSRLLAIQTTQEMPGRALINVYGPTECTINSSSYAVDPAELGEAPQSISIGAPVADTEYHILGKEDLKPVGVGEIGELYIGGGQLARGYLHRPDLTAERFLEIEVTEGAGPVRLYKTGDLGQWNPDGTVQFAGRADNQVKLRGYRVELDEISLAIENHDWVRNAAVIVKNDGRTGFQNLIACVELSEKEAALMDQGNHGSHHASKKSKLQVKAQLSNPGLRDDADLAARVAYDLPGAEPTPEQRSRVFARKTYRFYEGGAVTEADLLALLGGQVPAAYSRKAADLAPAELGQILRWFGQYLSEERLLPKYGYASPGALYATQLYFELEGVGGLQPGYYYYQPQRHQLVLISEKAATGRPTAHIHFIGKRGGIEPVYKNNIQEVLEIETGHIVGLFEQVLPAYGLDIRDLAYEPAVRDLLDVPEEDFYLGTFELVPHTGRREDHAEVYVQTHGSKVANLPEGQYRYADGTLTRFSDDIVLKKQVIAINQSVYQAASFGISVISRAPEEWMHYVTLGKKLQHLMMNGLGLGFMSSGYSSKTGNPLPASRRIDSVLQANGVESGPSYFFVGGRVSDEQLGHEGMREDSVHMRGPAELIRDDLVSFLPDYMIPNRVVVFERLPLSANGKIDAKALAASDQVNAELVERPFVAPRTETEKEIAEVWAKSLRRESVSVQDDFFESGGNSLIAVGLIRELNSRLGVSLPLQSVLESPTVEKLSRRLEREVAQESSRLVRLHAETGKDRPVLCWPGLGGYPMNLRTLAGEIGLGRSFYGIQAHGINEGEAPYATITEMAKADIEAIKELQPKGPYTLWGYSFGARVAFETAYQLEQAGEKVDNLFLIAPGSPTVRAENGKVYGREASFANRAYTTILFSVFTGTISGPDLEKCLESATDEESFAGFISELKGIDVDLAKRIISVVGQTYEFEYSFRELAERTLAAPVTIFKARGDDYSFIENSNGYSAEPPTVIDLDADHYSLLRTPDIGELVKHIRYLLGE

SEQ ID NO: 5 - DNA, 2934 bp, 现代玫瑰(Rosa hybrida)
aagcttcagcaagagttgaagaaatagggacagagccatccatgtgctttgatgaatctgatgggatacaaaatgtgaaagattcacttgctgatttatccagaatttcttcatatagtgaggagaatgttgaaagatctaatgatgagcactctgttaaactagacggaattcatgtgcagcacgagtgtcatgagggcagtgaagaagacaaacctgatggtaagagcggtgagaatgcagttgatctggctaatcatggcatggctcgaactgatttttgtcagataacagaagagattgagaatggagtagtcatcactgagatgagcaacattgccaaccctgataaaactgatattccaaacggggtgcctcaaaatgagactgatgatggatttaataacactcaggatgatgctaatacaaaggaagtgacagaagagaattctgacagacgtgcgaaggaagtgacagaagagaattctgacaaagatgttttgaagaatatccttgaattctcacgtgcttcttctgtggtggattttgaaattccagtgttggatgtgaaatttacttctcttgaaagttgcagtgccacttgttctcttgcagcccttttgtctgaatcgccggaatcaatgactgaagcaccttgtgtgaggcaaattgatgatgtgcccccggttggtgaggagtctagcttgattttggtggaagatcgggagccggttggtcctactcctgatggtaatttttctgtggatatggattactatagtgtagcagaacctttgagcacatgggatgcgaatctgcagtgtgaaacatcaaatagccatgagacttttgctgcaagtctcatttgatagcttctgtgttaataactttgttagtctgtacataaatttgtctagacaagaattggtcgtgtactatcgtgtgtttttgccgtgctttagtactcatgaaccaattcagagaaaactggctgcatattttgaggagtctctgaattcttcaatgctcaactggtatgcatgtaggtggcatatcacttcagggattcttctattctttaactttacgcatcttgacattttgtatataacaaaatcaggtctattgggtgaaagtaattggctagaatggaaagctctacggttttaccgcaggtcaattttcatagctccacaagtgaattgaaaatgctcataggctttatgtttgtcctccacctctggcgacgatgtttgttggggagttaactcaaacctaccaccaaactcgaacccatcttccataatttataatacaaatttgcgatcatttgttcatccaattattgtgacactcggctaccacccaaaatatcggtcacagacccaaacgtattgtcacaacaaatcgtgtctctcgcattaaacacagctagaaagaagagttgaacccacaattcgagcacccactacctatgtacgaagtcatgagttcgagtcaccataggggtagaagtgaaatcatttgatcatctttaaagaaataaaaggaagagttgaacccacaattggctcttgtcccaaaaagaactaatagttcagtgcaccgacgtgtatttgcaccgacataaatggattgttagattatattaaatacactcttaggttattaataaaaatattaattataaatatcaaaagttgagatcatcttataaatgttgggtcagttacaccgtcggtgcatagaataatttccaaactatataatagccttcattttctgatttagctcatgggacatgattgctataaataattgtactcgtagaggcatacttgtgtctttttatacagttgtactgaagctcagaaaagtttatgaaggtgagaactgagaagggcaaggcatttggtagttgaggtatatgagagcatgaaccccatgcattgcagctaccacctctcttttttccttcttcccatacaaataaaaccaactcttctcacctaagtctatcatctttatttatggcagctcttgcttaattagctcatctatattatattatttatctataatatgtgtcactctgtctacctaccagcccaaaataaaactgataatagtcaatttgatgatattttttgttttttgttttgttttgtcttttttgtattgatttttttaaaattaaaatgacttcattttttgtttttgtttttttttctatttttttttatagaaaaattggcaaactttcattatctgttattgatgacaattaagccattaaaacctataattaattatctttcaattcgagtaaatttaaaacggtgtaaaattaaaatatgatcgtattcttaaatgaataaaactcacttaataatagtaatacttgaatcacatctacgaacatagattcttttcatccagtctaaccatgtttgaatatatagagtttgattatggttatgtctttgtccacattttggtttgtaaataaatgtgcaacggaggtatggtactgttgctctatcaaattcaagtttgaattaaaagaaaaaaaaaaagacgatattttgtgcgctttgtttggtaggtaaaacgagagaacaaacgcattccaaatcatgcggattttgatcggcaacacacaccacaaaaaaccgtacacgatgcacgtgccatttgccgggggtttctaacaaggtaattgggcaggcacgtgatcccccagctacccacctctcgcttcccttctcaaactccttttccatgtatatatacaaccccttttctcagaccattatattctaacatttttgctttgctattgtaacgcaacaaaaactgctcattccatccttgttcctccccattttgatcttctctcgacccttctccgagatgggtaccgagctcgaattc

SEQ ID NO: 6 - DNA, 1183 bp, 现代玫瑰(Rosa hybrida)
cgatggactccagagcggccgcggggtgggtttccccaccacgtgtctttacgaccctccaatcagaagagaggaaattttcaatcttttccaaaattgcccctgctccctgaagtgcaatacccaaaacactcccctgctgggcattgattggccctccccaccacgtgtccgtgcgggtgccctacgcaagattctctcctcttcctcctctatatcccatcaatcattcacaggtaaaagaattaatgtatatctttgataaaataaatgagtaaaaactggacggttgatggaccctgaatcaaatgagtgattcccatggtttctctttacttttgcttcaggtccaatacaaaatgtattataccacttacatttccttgtaataataactaaagtcatatacattaaaaattgaagccaagttttggaaattagtataatggaggaaagatcgtttttccctttataaataccttctctgagtcccccttgctttcatttttctgcatatcttcttgtttagattgtggaaaagaaaagaagtctaagaaaaaacccaaaaggtagaaacctctctgtttctttcatcatctccatcttctctttgttttcttatctgggtattgatcaaaatactcaaaacaccatctggtaatccaatcttcagtgcctcacttttttagtccaattcatgtttttgacttttgagtactccacagctagctagatcagcaactgcttgatgtttgctgtcaaagaacccaaaaagcaatgaacttaaaattttttagtccatcagttcacaatttcttttagtccaattcatgtttttagctccacagctagatcagcaactgtactttgatgtttgttgtcaaagaacccaaagtgcaatgaacttattaactctcagtccatcagttcgcaatttcttgagctagttagctagttgtagtgtaacaccacgcttttcttgatcaaagctagataggggagattagtactatttagaaaccgtcttttgattttctaatttgtacataaagtttgatccttttttgcttgattgatgattctcattgtacattggccttttttttttctttcccctacttgattgatgactctcattgtggaaaagaaaagaagtctaagaaaaaacccaaaagctgcaact

SEQ ID NO: 7 - DNA, 4491 bp, 人工序列(Artificial Sequence)
tgaaggcgggaaacgacaatctgatcatgagcggagaattaagggagtcacgttatgacccccgccgatgacgcgggacaagccgttttacgtttggctcgaggataatttatttgaaaattcataagaaaagcaaacgttacatgaattgatgaaacaatacaaagacagataaagccacgcacatttaggatattggccgagattactgaatattgagtaagatcacggaatttctgacaggagcatgtcttcaattcagcccaaatggcagttgaaatactcaaaccgccccatatgcaggagcggatcattcattgtttgtttggttgcctttgccaacatgggagtccaagggatccgaattcgagctcggtacccatctcggagaagggtcgagagaagatcaaaatggggaggaacaaggatggaatgagcagtttttgttgcgttacaatagcaaagcaaaaatgttagaatataatggtctgagaaaaggggttgtatatatacatggaaaaggagtttgagaagggaagcgagaggtgggtagctgggggatcacgtgcctgcccaattaccttgttagaaacccccggcaaatggcacgtgcatcgtgtacggttttttgtggtgtgtgttgccgatcaaaatccgcatgatttggaatgcgtttgttctctcgttttacctaccaaacaaagcgcacaaaatatcgtctttttttttttcttttaattcaaacttgaatttgatagagcaacagtaccatacctccgttgcacatttatttacaaaccaaaatgtggacaaagacataaccataatcaaactctatatattcaaacatggttagactggatgaaaagaatctatgttcgtagatgtgattcaagtattactattattaagtgagttttattcatttaagaatacgatcatattttaattttacaccgttttaaatttactcgaattgaaagataattaattataggttttaatggcttaattgtcatcaataacagataatgaaagtttgccaatttttctataaaaaaaaatagaaaaaaaaacaaaaacaaaaaatgaagtcattttaattttaaaaaaatcaatacaaaaaagacaaaacaaaacaaaaaacaaaaaatatcatcaaattgactattatcagttttattttgggctggtaggtagacagagtgacacatattatagataaataatataatatagatgagctaattaagcaagagctgccataaataaagatgatagacttaggtgagaagagttggttttatttgtatgggaagaaggaaaaaagagaggtggtagctgcaatgcatggggttcatgctctcatatacctcaactaccaaatgccttgcccttctcagttctcaccttcataaacttttctgagcttcagtacaactgtataaaaagacacaagtatgcctctacgagtacaattatttatagcaatcatgtcccatgagctaaatcagaaaatgaaggctattatatagtttggaaattattctatgcaccgacggtgtaactgacccaacatttataagatgatctcaacttttgatatttataattaatatttttattaataacctaagagtgtatttaatataatctaacaatccatttatgtcggtgcaaatacacgtcggtgcactgaactattagttctttttgggacaagagccaattgtgggttcaactcttccttttatttctttaaagatgatcaaatgatttcacttctacccctatggtgactcgaactcatgacttcgtacataggtagtgggtgctcgaattgtgggttcaactcttctttctagctgtgtttaatgcgagagacacgatttgttgtgacaatacgtttgggtctgtgaccgatattttgggtggtagccgagtgtcacaataattggatgaacaaatgatcgcaaatttgtattataaattatggaagatgggttcgagtttggtggtaggtttgagttaactccccaacaaacatcgtcgccagaggtggaggacaaacataaagcctatgagcattttcaattcacttgtggagctatgaaaattgacctgcggtaaaaccgtagagctttccattctagccaattactttcacccaatagacctgattttgttatatacaaaatgtcaagatgcgtaaagttaaagaatagaagaatccctgaagtgatatgccacctacatgcataccagttgagcattgaagaattcagagactcctcaaaatatgcagccagttttctctgaattggttcatgagtactaaagcacggcaaaaacacacgatagtacacgaccaattcttgtctagacaaatttatgtacagactaacaaagttattaacacagaagctatcaaatgagacttgcagcaaaagtctcatggctatttgatgtttcacactgcagattcgcatcccatgtgctcaaaggttctgctacactatagtaatccatatccacagaaaaattaccatcaggagtaggaccaaccggctcccgatcttccaccaaaatcaagctagactcctcaccaaccgggggcacatcatcaatttgcctcacacaaggtgcttcagtcattgattccggcgattcagacaaaagggctgcaagagaacaagtggcactgcaactttcaagagaagtaaatttcacatccaacactggaatttcaaaatccaccacagaagaagcacgtgagaattcaaggatattcttcaaaacatctttgtcagaattctcttctgtcacttccttcgcacgtctgtcagaattctcttctgtcacttcctttgtattagcatcatcctgagtgttattaaatccatcatcagtctcattttgaggcaccccgtttggaatatcagttttatcagggttggcaatgttgctcatctcagtgatgactactccattctcaatctcttctgttatctgacaaaaatcagttcgagccatgccatgattagccagatcaactgcattctcaccgctcttaccatcaggtttgtcttcttcactgccctcatgacactcgtgctgcacatgaattccgtctagtttaacagagtgctcatcattagatctttcaacattctcctcactatatgaagaaattctggataaatcagcaagtgaatctttcacattttgtatcccatcagattcatcaaagcacatggatggctctgtccctatttcttcaactcttgctgaagcttcccgggcgatggactccagagcggccgcggggtgggtttccccaccacgtgtctttacgaccctccaatcagaagagaggaaattttcaatcttttccaaaattgcccctgctccctgaagtgcaatacccaaaacactcccctgctgggcattgattggccctccccaccacgtgtccgtgcgggtgccctacgcaagattctctcctcttcctcctctatatcccatcaatcattcacaggtaaaagaattaatgtatatctttgataaaataaatgagtaaaaactggacggttgatggaccctgaatcaaatgagtgattcccatggtttctctttacttttgcttcaggtccaatacaaaatgtattataccacttacatttccttgtaataataactaaagtcatatacattaaaaattgaagccaagttttggaaattagtataatggaggaaagatcgtttttccctttataaataccttctctgagtcccccttgctttcatttttctgcatatcttcttgtttagattgtggaaaagaaaagaagtctaagaaaaaacccaaaaggtagaaacctctctgtttctttcatcatctccatcttctctttgttttcttatctgggtattgatcaaaatactcaaaacaccatctggtaatccaatcttcagtgcctcacttttttagtccaattcatgtttttgacttttgagtactccacagctagctagatcagcaactgcttgatgtttgctgtcaaagaacccaaaaagcaatgaacttaaaattttttagtccatcagttcacaatttcttttagtccaattcatgtttttagctccacagctagatcagcaactgtactttgatgtttgttgtcaaagaacccaaagtgcaatgaacttattaactctcagtccatcagttcgcaatttcttgagctagttagctagttgtagtgtaacaccacgcttttcttgatcaaagctagataggggagattagtactatttagaaaccgtcttttgattttctaatttgtacataaagtttgatccttttttgcttgattgatgattctcattgtacattggccttttttttttctttcccctacttgattgatgactctcattgtggaaaagaaaagaagtctaagaaaaaacccaaaagctgcaactactagt

SEQ ID NO: 8 - DNA, 48 bp, 人工序列(Artificial Sequence)
agaaaaaacccaaaagctgcaactaatgacccttcaagaaaccagcgt

SEQ ID NO: 9 - DNA, 55 bp, 人工序列(Artificial Sequence)
ttgaacgatcggggaaattcgagctcattattcacccagcagatagcgaatatgt

SEQ ID NO: 10 - DNA, 57 bp, 人工序列(Artificial Sequence)
gagatgggtaccgagctcgaattcgatgaagatttacagaatttatatggaccgccc

SEQ ID NO: 11 - DNA, 55 bp, 人工序列(Artificial Sequence)
cctttgccaacatgggagtccaaggctataaaagctcttcgtacgacaccattgt